European Patent Application EP 4 563 559 A1, published June 4, 2025. Title: チオ化溶液. Applicant: SUMITOMO CHEMICAL COMPANY, LIMITED. The sequence listing filed with the application follows.

SEQUENCE LISTING (10 sequences)

SEQ ID NO: 1 - RNA, 21 nt, synthetic construct
  misc_feature 1..21
  modified_base join(7,17): mod_base = um
  source 1..21: mol_type = other RNA
atggaanactcttggtnacnn

SEQ ID NO: 2 - RNA, 21 nt, synthetic construct
  misc_feature 1..21: note = Synthetic oligonucleotide
  misc_feature join(2,12,14..15,19): note = modified base - um
  misc_feature join(5..6,16..17): note = modified base - cm
  misc_feature 20..21: note = modified base - dT
  source 1..21: mol_type = other RNA
gnaannaagagnannnnannn

SEQ ID NO: 3 - RNA, 36 nt, synthetic construct
  misc_feature 1..36: note = Synthetic oligonucleotide
  source 1..36: mol_type = other RNA
agagccagccttcttattgttttagagctatgctgt

SEQ ID NO: 4 - RNA, 67 nt, synthetic construct
  misc_feature 1..67: note = Synthetic oligonucleotide
  source 1..67: mol_type = other RNA
acagcatagcaagttaaaataaggctagtccgttatcaacttgaaaaagtggcaccgagtcggtgct

SEQ ID NO: 5 - RNA, 94 nt, synthetic construct
  misc_feature 1..94: note = Synthetic oligonucleotide
  source 1..94: mol_type = other RNA
gttttcccttttcaaagaaatctcctgggcacctatcttcttaggtgccctcccttgtttaaacctgaccagttaaccggctggttaggttttt

SEQ ID NO: 6 - RNA, 100 nt, synthetic construct
  misc_feature 1..100: note = Synthetic oligonucleotide
  source 1..100: mol_type = other RNA
agtcctcatctccctcaagcgttttagagctagtaatagcaagttaaaataaggctagtccgttatcaacttgaaaaagtggcaccgagtcggtgctttt

SEQ ID NO: 7 - RNA, 113 nt, synthetic construct
  misc_feature 1..113: note = Synthetic oligonucleotide
  source 1..113: mol_type = other RNA
gcagatgtagtgtttccacagtttaagagctatgctggaaacagcatagcaagtttaaataaggctagtccgttatcaacttgaaaaagtggcaccgagtcggtgcttttttt

SEQ ID NO: 8 - RNA, 113 nt, synthetic construct
  misc_feature 1..113: note = Synthetic oligonucleotide
  misc_feature join(1,8,17..18): note = modified base - dA
  misc_feature join(2,19): note = modified base - dG
  misc_feature join(3,6,9,11,15): note = modified base - dT
  misc_feature join(4..5,7,10,12..14,16,20): note = modified base - dC
  source 1..113: mol_type = other RNA
nnnnnnnnnnnnnnnnnnnngtttaagagctatgctggtaacagcatagcaagtttaaataaggctagtccgttatcaacttgaaaaagtggcaccgagtcggtgcttttttt

SEQ ID NO: 9 - RNA, 113 nt, synthetic construct
  misc_feature 1..113: note = Synthetic oligonucleotide
  misc_feature 1: note = modified base - am
  misc_feature 2: note = modified base - gm
  misc_feature join(3,110..112): note = modified base - um
  misc_feature join(1..4,110..113): note = phosphorothioate modification
  source 1..113: mol_type = other RNA
nnncctcatctccctcaagcgtttaagagctatgctggtaacagcatagcaagtttaaataaggctagtccgttatcaacttgaaaaagtggcaccgagtcggtgctttnnnt

SEQ ID NO: 10 - RNA, 100 nt, synthetic construct
  misc_feature 1..100: note = Synthetic oligonucleotide
  misc_feature 1: note = modified base - am
  misc_feature 2: note = modified base - cm
  misc_feature join(3,97..99): note = modified base - um
  misc_feature join(1..4,97..100): note = phosphorothioate modification
  source 1..100: mol_type = other RNA
nnncaatttgtaaaaaagttttagagctagaaatagcaagttaaaataaggctagtccgttatcaacttgaaaaagtggcaccgagtcggtgctttnnnt